European Patent Specification EP 4 021 415 B1, published May 14, 2025. Title: CANNABINOID CONTAINING TARGETING LIPOSOMES. Applicant: NEXTAGE CANNABIS INNOVATION LTD. The sequence listing filed with the application follows.

SEQUENCE LISTING (1 sequence)

SEQ ID NO: 1 - protein, 7 aa, Artificial Sequence
  Synthetic polypeptide
  MISC_FEATURE (6)..(6): Optionally M is oxidized or methionine sulfoxide
AHRERMS